European Patent Specification EP 3 665 189 B1, published November 6, 2024. Title: Fc binding proteins with Cysteine in helix 3. Applicant: Navigo Proteins GmbH. The sequence listing filed with the application follows.

SEQUENCE LISTING (99 sequences)

SEQ ID NO: 1 - protein, 58 aa, Artificial Sequence
  consensus sequence 1
  variant (1)..(1): may be replaced by A, N, Q, V, or deleted
  variant (2)..(2): may be replaced by D or Q, or deleted
  variant (3)..(3): may be replaced by N, or deleted
  variant (4)..(4): may be replaced by Q or N, or deleted
  variant (5)..(5): may be replaced by F, or deleted
  variant (6)..(6): may be replaced by N, or deleted
  variant (7)..(7): may be replaced by E
  variant (8)..(8): may be replaced by A or E
  variant (11)..(11): may be replaced by S, N, I ,or E
  variant (15)..(15): may be replaced by Q
  variant (16)..(16): may be replaced by V
  variant (18)..(18): may be replaced by N
  variant (19)..(19): may be replaced by M
  variant (23)..(23): may be replaced by N
  variant (24)..(24): may be replaced by A
  variant (25)..(25): may be replaced by E
  variant (29)..(29): may be replaced by G
  variant (35)..(35): may be replaced by K or I
  variant (40)..(40): may be replaced by Q or T
  variant (42)..(42): may be replaced by A, K, or T
  variant (43)..(43): may be replaced by S, N, or C
  variant (44)..(44): may be replaced by L or V
  variant (46)..(46): may be replaced by C or A
  variant (47)..(47): may be replaced by C
  variant (49)..(49): may be replaced by Q
  variant (50)..(50): may be replaced by C
  variant (51)..(51): may be replaced by C
  variant (53)..(53): may be replaced by E or C
  variant (54)..(54): may be replaced by S, or deleted
  variant (57)..(57): may be deleted
  variant (58)..(58): may be replaced by K, or deleted
IAAKHDKDQQAAFYEILHLPNLTEDQRNAFIQSLRDDPSVSLEILGEAKKLNDAQAPP

SEQ ID NO: 2 - protein, 58 aa, Artificial Sequence; identical to SEQ ID NO: 1
  consensus sequence 2
  variant (1)..(1): may be deleted
  variant (2)..(2): may be replaced by D, or deleted
  variant (3)..(3): may be replaced by N or deleted
  variant (4)..(4): may be replaced by Q, or deleted
  variant (5)..(5): may be replaced by F, or deleted
  variant (6)..(6): may be deleted
  variant (7)..(7): may be replaced by E
  variant (8)..(8): may be replaced by A or E
  variant (11)..(11): may be replaced by S, I, or E
  variant (25)..(25): may be replaced by E
  variant (35)..(35): may be replaced by I
  variant (40)..(40): may be replaced by Q or T
  variant (43)..(43): may be replaced by S, or C
  variant (44)..(44): may be replaced by L or V
  variant (46)..(46): may be replaced by C or A
  variant (47)..(47): may be replaced by C
  variant (49)..(49): may be replaced by Q
  variant (50)..(50): may be replaced by C
  variant (51)..(51): may be replaced by  C
  variant (53)..(53): may be replaced by E or C
  variant (54)..(54): may be replaced by S
  variant (57)..(57): may be deleted
  variant (58)..(58): may be replaced by K, or deleted

SEQ ID NO: 3 - protein, 58 aa, Artificial Sequence; identical to SEQ ID NO: 1
  cs14

SEQ ID NO: 4 - protein, 58 aa, Artificial Sequence
  cs27
IAAKFDEAQQAAFYEILHLPNLTEEQRNAFIQSLRDDPSVSLEVLGEAQKLNDSQAPK

SEQ ID NO: 5 - protein, 58 aa, Artificial Sequence
  cs20
IDSKFDEAQQAAFYEILHLPSLTEDQRNAFIQSLRDDPSTSLSLLGEAKKLNDAQAPP

SEQ ID NO: 6 - protein, 58 aa, Artificial Sequence
  cs42
IDAKHDEDQQAAFYEILHLPNLTEEQRNAFIQSLRDDPSQSLEILGEAKKLNESQAPK

SEQ ID NO: 7 - protein, 58 aa, Artificial Sequence
  cs26
IAAQHDKDQQAAFYEILHLPNLTEEQRNAFIQSLRDDPSVSLEILAEAKKLNDAQAPK

SEQ ID NO: 8 - protein, 58 aa, Artificial Sequence
  cs24
IAAQHDKEQQAAFYEILHLPNLTEDQRNAFIQSLRDDPSVSLEILGEAKKLNDAQAPK

SEQ ID NO: 9 - protein, 58 aa, Artificial Sequence
  cs17
IDSKFDEAQQAAFYEILHLPNLTEDQRNAFIQSLRDDPSVSLSLLGEAKKLNDAQAPP

SEQ ID NO: 10 - protein, 58 aa, Artificial Sequence
  cs25
IAAKHDKDQQAAFYEILHLPNLTEDQRNAFIQSLRDDPSVSLEILAEAKKLNDAQAPK

SEQ ID NO: 11 - protein, 58 aa, Artificial Sequence
  cs47h3
IAAKHDKDQQAAFYEILHLPNLTEDQRNAFIQSLRDDPSVSLEVLGEAQKLNDSQAPK

SEQ ID NO: 12 - protein, 58 aa, Artificial Sequence
  cs47h4
IAAKHDKDQQAAFYEILHLPNLTEEQRNAFIQSLRDDPSVSLEVLGEAQKLNDSQAPK

SEQ ID NO: 13 - protein, 58 aa, Artificial Sequence
  cs74h1
IAAKFDEAQQAAFYEILHLPNLTEDQRNAFIQSLRDDPSVSLEILGEAKKLNDAQAPP

SEQ ID NO: 14 - protein, 58 aa, Artificial Sequence
  cs74h2
IAAKFDEAQQAAFYEILHLPNLTEEQRNAFIQSLRDDPSVSLEILGEAKKLNDAQAPP

SEQ ID NO: 15 - protein, 58 aa, Artificial Sequence
  cs41
IAAKHDEDQQAAFYEILHLPNLTEEQRNAFIQSLRDDPSVSLEILGEAKKLNDSQAPK

SEQ ID NO: 16 - protein, 58 aa, Artificial Sequence
  cs43
IAAKHDKDQQAAFYEILHLPNLTEEQRNAFIQSLRDDPSVSLEILGEAKKLNDSQAPK

SEQ ID NO: 17 - protein, 58 aa, Artificial Sequence
  cs14 43C
IAAKHDKDQQAAFYEILHLPNLTEDQRNAFIQSLRDDPSVSLCILGEAKKLNDAQAPP

SEQ ID NO: 18 - protein, 58 aa, Artificial Sequence
  cs14 46C
IAAKHDKDQQAAFYEILHLPNLTEDQRNAFIQSLRDDPSVSLEILCEAKKLNDAQAPP

SEQ ID NO: 19 - protein, 58 aa, Artificial Sequence
  cs14 47C
IAAKHDKDQQAAFYEILHLPNLTEDQRNAFIQSLRDDPSVSLEILGCAKKLNDAQAPP

SEQ ID NO: 20 - protein, 58 aa, Artificial Sequence
  cs14 11S 46C
IAAKHDKDQQSAFYEILHLPNLTEDQRNAFIQSLRDDPSVSLEILCEAKKLNDAQAPP

SEQ ID NO: 21 - protein, 58 aa, Artificial Sequence
  cs27 43C
IAAKFDEAQQAAFYEILHLPNLTEEQRNAFIQSLRDDPSVSLCVLGEAQKLNDSQAPK

SEQ ID NO: 22 - protein, 58 aa, Artificial Sequence
  cs27 46C
IAAKFDEAQQAAFYEILHLPNLTEEQRNAFIQSLRDDPSVSLEVLCEAQKLNDSQAPK

SEQ ID NO: 23 - protein, 58 aa, Artificial Sequence
  cs27 47C
IAAKFDEAQQAAFYEILHLPNLTEEQRNAFIQSLRDDPSVSLEVLGCAQKLNDSQAPK

SEQ ID NO: 24 - protein, 58 aa, Artificial Sequence
  cs27 11S 46C
IAAKFDEAQQSAFYEILHLPNLTEEQRNAFIQSLRDDPSVSLEVLCEAQKLNDSQAPK

SEQ ID NO: 25 - protein, 116 aa, Artificial Sequence
  cs27 46C dimer
IAAKFDEAQQAAFYEILHLPNLTEEQRNAFIQSLRDDPSVSLEVLCEAQKLNDSQAPKIAAKFDEAQQAAFYEILHLPNLTEEQRNAFIQSLRDDPSVSLEVLCEAQKLNDSQAPK

SEQ ID NO: 26 - protein, 58 aa, Artificial Sequence
  cs26 43C
IAAQHDKDQQAAFYEILHLPNLTEEQRNAFIQSLRDDPSVSLCILAEAKKLNDAQAPK

SEQ ID NO: 27 - protein, 58 aa, Artificial Sequence
  cs26 46C
IAAQHDKDQQAAFYEILHLPNLTEEQRNAFIQSLRDDPSVSLEILCEAKKLNDAQAPK

SEQ ID NO: 28 - protein, 58 aa, Artificial Sequence
  cs26 47C
IAAQHDKDQQAAFYEILHLPNLTEEQRNAFIQSLRDDPSVSLEILACAKKLNDAQAPK

SEQ ID NO: 29 - protein, 58 aa, Artificial Sequence
  cs26 11S 46C
IAAQHDKDQQSAFYEILHLPNLTEEQRNAFIQSLRDDPSVSLEILCEAKKLNDAQAPK

SEQ ID NO: 30 - protein, 58 aa, Artificial Sequence
  cs26 9H 46C
IAAQHDKDHQAAFYEILHLPNLTEEQRNAFIQSLRDDPSVSLEILCEAKKLNDAQAPK

SEQ ID NO: 31 - protein, 58 aa, Artificial Sequence
  cs26 36H 46C
IAAQHDKDQQAAFYEILHLPNLTEEQRNAFIQSLRHDPSVSLEILCEAKKLNDAQAPK

SEQ ID NO: 32 - protein, 116 aa, Artificial Sequence
  cs26 46C dimer
IAAQHDKDQQAAFYEILHLPNLTEEQRNAFIQSLRDDPSVSLEILCEAKKLNDAQAPKIAAQHDKDQQAAFYEILHLPNLTEEQRNAFIQSLRDDPSVSLEILCEAKKLNDAQAPK

SEQ ID NO: 33 - protein, 55 aa, Artificial Sequence
  cs26 delN 46C
AHDKDQQAAFYEILHLPNLTEEQRNAFIQSLRDDPSVSLEILCEAKKLNDAQAPK

SEQ ID NO: 34 - protein, 53 aa, Artificial Sequence
  cs26 delNC 46C
QHDKDQQAAFYEILHLPNLTEEQRNAFIQSLRDDPSVSLEILCEAKKLNDAQA

SEQ ID NO: 35 - protein, 174 aa, Artificial Sequence
  cs26 46C trimer
IAAQHDKDQQAAFYEILHLPNLTEEQRNAFIQSLRDDPSVSLEILCEAKKLNDAQAPKIAAQHDKDQQAAFYEILHLPNLTEEQRNAFIQSLRDDPSVSLEILCEAKKLNDAQAPKIAAQHDKDQQAAFYEILHLPNLTEEQRNAFIQSLRDDPSVSLEILCEAKKLNDAQAPK

SEQ ID NO: 36 - protein, 58 aa, Artificial Sequence
  cs24 43C
IAAQHDKEQQAAFYEILHLPNLTEDQRNAFIQSLRDDPSVSLCILGEAKKLNDAQAPK

SEQ ID NO: 37 - protein, 58 aa, Artificial Sequence
  cs24 46C
IAAQHDKEQQAAFYEILHLPNLTEDQRNAFIQSLRDDPSVSLEILCEAKKLNDAQAPK

SEQ ID NO: 38 - protein, 58 aa, Artificial Sequence
  cs24 47C
IAAQHDKEQQAAFYEILHLPNLTEDQRNAFIQSLRDDPSVSLEILGCAKKLNDAQAPK

SEQ ID NO: 39 - protein, 58 aa, Artificial Sequence
  cs24 11S 46C
IAAQHDKEQQSAFYEILHLPNLTEDQRNAFIQSLRDDPSVSLEILCEAKKLNDAQAPK

SEQ ID NO: 40 - protein, 58 aa, Artificial Sequence
  cs47h3 43C
IAAKHDKDQQAAFYEILHLPNLTEDQRNAFIQSLRDDPSVSLCVLGEAQKLNDSQAPK

SEQ ID NO: 41 - protein, 58 aa, Artificial Sequence
  cs47h3 46C
IAAKHDKDQQAAFYEILHLPNLTEDQRNAFIQSLRDDPSVSLEVLCEAQKLNDSQAPK

SEQ ID NO: 42 - protein, 58 aa, Artificial Sequence
  cs47h3 47C
IAAKHDKDQQAAFYEILHLPNLTEDQRNAFIQSLRDDPSVSLEVLGCAQKLNDSQAPK

SEQ ID NO: 43 - protein, 58 aa, Artificial Sequence
  cs47h3 11S 46C
IAAKHDKDQQSAFYEILHLPNLTEDQRNAFIQSLRDDPSVSLEVLCEAQKLNDSQAPK

SEQ ID NO: 44 - protein, 58 aa, Artificial Sequence
  cs47h4 43C
IAAKHDKDQQAAFYEILHLPNLTEEQRNAFIQSLRDDPSVSLCVLGEAQKLNDSQAPK

SEQ ID NO: 45 - protein, 58 aa, Artificial Sequence
  cs47h4 46C
IAAKHDKDQQAAFYEILHLPNLTEEQRNAFIQSLRDDPSVSLEVLCEAQKLNDSQAPK

SEQ ID NO: 46 - protein, 58 aa, Artificial Sequence
  cs47h4 47C
IAAKHDKDQQAAFYEILHLPNLTEEQRNAFIQSLRDDPSVSLEVLGCAQKLNDSQAPK

SEQ ID NO: 47 - protein, 58 aa, Artificial Sequence
  cs74h1 43C
IAAKFDEAQQAAFYEILHLPNLTEDQRNAFIQSLRDDPSVSLCILGEAKKLNDAQAPP

SEQ ID NO: 48 - protein, 58 aa, Artificial Sequence
  cs74h1 46C
IAAKFDEAQQAAFYEILHLPNLTEDQRNAFIQSLRDDPSVSLEILCEAKKLNDAQAPP

SEQ ID NO: 49 - protein, 58 aa, Artificial Sequence
  cs74h1 47C
IAAKFDEAQQAAFYEILHLPNLTEDQRNAFIQSLRDDPSVSLEILGCAKKLNDAQAPP

SEQ ID NO: 50 - protein, 58 aa, Artificial Sequence
  cs74h2 43C
IAAKFDEAQQAAFYEILHLPNLTEEQRNAFIQSLRDDPSVSLCILGEAKKLNDAQAPP

SEQ ID NO: 51 - protein, 58 aa, Artificial Sequence
  cs74h2 46C
IAAKFDEAQQAAFYEILHLPNLTEEQRNAFIQSLRDDPSVSLEILCEAKKLNDAQAPP

SEQ ID NO: 52 - protein, 58 aa, Artificial Sequence
  cs74h2 47C
IAAKFDEAQQAAFYEILHLPNLTEEQRNAFIQSLRDDPSVSLEILGCAKKLNDAQAPP

SEQ ID NO: 53 - protein, 58 aa, Artificial Sequence
  cs20 46C
IDSKFDEAQQAAFYEILHLPSLTEDQRNAFIQSLRDDPSTSLSLLCEAKKLNDAQAPP

SEQ ID NO: 54 - protein, 58 aa, Artificial Sequence
  cs20 43C
IDSKFDEAQQAAFYEILHLPSLTEDQRNAFIQSLRDDPSTSLCLLGEAKKLNDAQAPP

SEQ ID NO: 55 - protein, 58 aa, Artificial Sequence
  cs20 47C
IDSKFDEAQQAAFYEILHLPSLTEDQRNAFIQSLRDDPSTSLSLLGCAKKLNDAQAPP

SEQ ID NO: 56 - protein, 58 aa, Artificial Sequence
  cs20 11S 46C
IDSKFDEAQQSAFYEILHLPSLTEDQRNAFIQSLRDDPSTSLSLLCEAKKLNDAQAPP

SEQ ID NO: 57 - protein, 58 aa, Artificial Sequence
  cs17 46C
IDSKFDEAQQAAFYEILHLPNLTEDQRNAFIQSLRDDPSVSLSLLCEAKKLNDAQAPP

SEQ ID NO: 58 - protein, 58 aa, Artificial Sequence
  cs42 46C
IDAKHDEDQQAAFYEILHLPNLTEEQRNAFIQSLRDDPSQSLEILCEAKKLNESQAPK

SEQ ID NO: 59 - protein, 58 aa, Artificial Sequence
  cs42 47C
IDAKHDEDQQAAFYEILHLPNLTEEQRNAFIQSLRDDPSQSLEILGCAKKLNESQAPK

SEQ ID NO: 60 - protein, 58 aa, Artificial Sequence
  cs42 43C
IDAKHDEDQQAAFYEILHLPNLTEEQRNAFIQSLRDDPSQSLCILGEAKKLNESQAPK

SEQ ID NO: 61 - protein, 58 aa, Artificial Sequence
  cs42 11S 46C
IDAKHDEDQQSAFYEILHLPNLTEEQRNAFIQSLRDDPSQSLEILCEAKKLNESQAPK

SEQ ID NO: 62 - protein, 58 aa, Artificial Sequence
  cs41 46C
IAAKHDEDQQAAFYEILHLPNLTEEQRNAFIQSLRDDPSVSLEILCEAKKLNDSQAPK

SEQ ID NO: 63 - protein, 58 aa, Artificial Sequence
  cs28 46C
IDAQHDEDQQAAFYEILHLPNLTEEQRNAFIQSLRDDPSQSLEILCEAKKLNESQAPK

SEQ ID NO: 64 - protein, 58 aa, Artificial Sequence
  cs23 46C
IAAKHDKDQQAAFYEILHLPSLTEDQRNAFIQSLRDDPSTSLSILCEAKKLNDAQAPP

SEQ ID NO: 65 - protein, 58 aa, Artificial Sequence
  cs25 46C
IAAKHDKDQQAAFYEILHLPNLTEDQRNAFIQSLRDDPSVSLEILCEAKKLNDAQAPK

SEQ ID NO: 66 - protein, 58 aa, Artificial Sequence
  cs31 46C
IAAKHDKDQQAAFYEILHLPSLTEDQRNAFIQSLRDDPSVSLEILCEAKKLDDAQAPK

SEQ ID NO: 67 - protein, 58 aa, Artificial Sequence
  cs43 46C
IAAKHDKDQQAAFYEILHLPNLTEEQRNAFIQSLRDDPSVSLEILCEAKKLNDSQAPK

SEQ ID NO: 68 - protein, 58 aa, Artificial Sequence
  cs44 46C
IAAKHDKDQQAAFYEILHLPNLTEEQRNAFIQSLRDDPSVSLEVLCEAKKLNDAQAPK

SEQ ID NO: 69 - protein, 58 aa, Artificial Sequence
  cs45 46C
IAAKHDKDQQAAFYEILHLPSLTEDARNAFIQSLRDDPSVSLEILCEAKKLDDAQAPK

SEQ ID NO: 70 - protein, 58 aa, Artificial Sequence
  cs15 46C
IDNKFDEAQQAAFYEILHLPNLTEDQRNAFIQSLRDDPSVSLEILCEAKKLNDAQAPP

SEQ ID NO: 71 - protein, 58 aa, Artificial Sequence
  cs16 46C
IDSKFDEAQQAAFYEILHLPNLTEDQRNAFIQSLRDDPSVSLEILCEAKKLNDAQAPP

SEQ ID NO: 72 - protein, 58 aa, Artificial Sequence
  cs35 46C
IDAKFDKEQQAAFYEILHLPNLTEEQRNAFIQSLRDDPSQSLELLCEAKKLNDAQAPK

SEQ ID NO: 73 - protein, 61 aa, Artificial Sequence
  cs17 11S 46C
IDSIDSKFDEAQQSAFYEILHLPNLTEDQRNAFIQSLRDDPSVSLSLLCEAKKLNDAQAPP

SEQ ID NO: 74 - protein, 58 aa, Artificial Sequence
  IB14 43C
PAAKHDKDQQSAFYEILHLPNLTEDQRSAFIQSLKDDPSVSKCILGEAKKLNDAQAPP

SEQ ID NO: 75 - protein, 58 aa, Artificial Sequence
  IB14 46C
PAAKHDKDQQSAFYEILHLPNLTEDQRSAFIQSLKDDPSVSKEILCEAKKLNDAQAPP

SEQ ID NO: 76 - protein, 58 aa, Artificial Sequence
  IB14 47C
PAAKHDKDQQSAFYEILHLPNLTEDQRSAFIQSLKDDPSVSKEILGCAKKLNDAQAPP

SEQ ID NO: 77 - protein, 58 aa, Artificial Sequence
  IB14 50C
PAAKHDKDQQSAFYEILHLPNLTEDQRSAFIQSLKDDPSVSKEILGEAKCLNDAQAPP

SEQ ID NO: 78 - protein, 58 aa, Artificial Sequence
  IB14
PAAKHDKDQQSAFYEILHLPNLTEDQRSAFIQSLKDDPSVSKEILGEAKKLNDAQAPP

SEQ ID NO: 79 - protein, 58 aa, Artificial Sequence
  IB27
AAAKFDEAQQSAFYEILHLPNLTEEQRNAFIQSLKDDPSVSKEVLGEAQKLNDSQAPK

SEQ ID NO: 80 - protein, 58 aa, Artificial Sequence
  IB24
AAAQHDKEQQSAFYEILHLPNLTEDQRNAFIQSLKDDPSVSKEILGEAKKLNDAQAPK

SEQ ID NO: 81 - protein, 58 aa, Artificial Sequence
  IB26
AAAQHDKDQQSAFYEILHLPNLTEEQRNAFIQSLKDDPSVSKEILAEAKKLNDAQAPK

SEQ ID NO: 82 - protein, 58 aa, Artificial Sequence
  IB28
ADAQHDEDQQSAFYEILHLPNLTEEQRNAFIQSLKDDPSQSKEILGEAKKLNESQAPK

SEQ ID NO: 83 - protein, 58 aa, Artificial Sequence
  IB20
ADAKFDEAQQSAFYEILHLPNLTEDQRNAFIQSLKDDPSTSKSLLGEAKKLNDAQAPP

SEQ ID NO: 84 - protein, 58 aa, Artificial Sequence
  domain C
ADNKFNKEQQNAFYEILHLPNLTEEQRNGFIQSLKDDPSVSKEILAEAKKLNDAQAPK

SEQ ID NO: 85 - protein, 58 aa, Artificial Sequence [sequence omitted]

SEQ ID NO: 86 - protein, 58 aa, Artificial Sequence [sequence omitted]

SEQ ID NO: 87 - protein, 10 aa, Artificial Sequence
  spacer
ASPAPSAPSA

SEQ ID NO: 88 - protein, 21 aa, Artificial Sequence
  spacer and taq
ASPAPSAPSACASWSHPQFEK

SEQ ID NO: 89 - protein, 8 aa, Artificial Sequence
  taq for purification
WSHPQFEK

SEQ ID NO: 90 - protein, 58 aa, Artificial Sequence
  cs26 50C
IAAQHDKDQQAAFYEILHLPNLTEEQRNAFIQSLRDDPSVSLEILAEAKCLNDAQAPK

SEQ ID NO: 91 - protein, 58 aa, Artificial Sequence
  cs26 51C
IAAQHDKDQQAAFYEILHLPNLTEEQRNAFIQSLRDDPSVSLEILAEAKKCNDAQAPK

SEQ ID NO: 92 - protein, 58 aa, Artificial Sequence
  cs26 53C
IAAQHDKDQQAAFYEILHLPNLTEEQRNAFIQSLRDDPSVSLEILAEAKKLNCAQAPK

SEQ ID NO: 93 - protein, 58 aa, Artificial Sequence
  cs24 50C
IAAQHDKEQQAAFYEILHLPNLTEDQRNAFIQSLRDDPSVSLEILGEAKCLNDAQAPK

SEQ ID NO: 94 - protein, 58 aa, Artificial Sequence
  cs24 51C
IAAQHDKEQQAAFYEILHLPNLTEDQRNAFIQSLRDDPSVSLEILGEAKKCNDAQAPK

SEQ ID NO: 95 - protein, 58 aa, Artificial Sequence
  cs24 53C
IAAQHDKEQQAAFYEILHLPNLTEDQRNAFIQSLRDDPSVSLEILGEAKKLNCAQAPK

SEQ ID NO: 96 - protein, 58 aa, Artificial Sequence
  cs26 40C
IAAQHDKDQQAAFYEILHLPNLTEEQRNAFIQSLRDDPSCSLEILAEAKKLNDAQAPK

SEQ ID NO: 97 - protein, 58 aa, Artificial Sequence
  cs26 42C
IAAQHDKDQQAAFYEILHLPNLTEEQRNAFIQSLRDDPSVSCEILAEAKKLNDAQAPK

SEQ ID NO: 98 - protein, 58 aa, Artificial Sequence
  cs26 49C
IAAQHDKDQQAAFYEILHLPNLTEEQRNAFIQSLRDDPSVSLEILAEACKLNDAQAPK

SEQ ID NO: 99 - protein, 58 aa, Artificial Sequence
  cs26 54C
IAAQHDKDQQAAFYEILHLPNLTEEQRNAFIQSLRDDPSVSLEILAEAKKLNDCQAPK